European Patent Specification EP 3 729 080 B1, published April 19, 2023. Title: Universal reporter cell assay for specificity test of novel antigen binding moieties. Applicant: F. Hoffmann-La Roche Ltd. The sequence listing filed with the application follows.

SEQUENCE LISTING (109 sequences)

SEQ ID NO: 1 - protein, 5 aa, Artificial sequence
  Anti-P329G CDR H1 Kabat
RYWMN

SEQ ID NO: 2 - protein, 17 aa, Artificial sequence
  Anti-P329G CDR H2 Kabat
EITPDSSTINYTPSLKD

SEQ ID NO: 3 - protein, 10 aa, Artificial sequence
  Anti-P329G CDR H3 Kabat
PYDYGAWFAS

SEQ ID NO: 4 - protein, 14 aa, Artificial sequence
  Anti-P329G CDR L1 Kabat
RSSTGAVTTSNYAN

SEQ ID NO: 5 - protein, 7 aa, Artificial sequence
  Anti-P329G CDR L2 Kabat
GTNKRAP

SEQ ID NO: 6 - protein, 9 aa, Artificial sequence
  Anti-P329G CDR L3 Kabat
ALWYSNHWV

SEQ ID NO: 7 - protein, 433 aa, Artificial sequence
  Anti-P329G-ds-scFv-CD28ATM-CD28CSD-CD3zSSD fusion pETR17096
EVKLLESGGGLVQPGGSLKLSCAASGFDFSRYWMNWVRQAPGKCLEWIGEITPDSSTINYTPSLKDKFIISRDNAKNTLYLQMIKVRSEDTALYYCVRPYDYGAWFASWGQGTLVTVSAGGGGSGGGGSGGGGSGGGGSQAVVTQESALTTSPGETVTLTCRSSTGAVTTSNYANWVQEKPDHLFTGLIGGTNKRAPGVPARFSGSLIGDKAALTITGAQTEDEAIYFCALWYSNHWVFGCGTKLTVLGGGGSFWVLVVVGGVLACYSLLVTVAFIIFWVRSKRSRLLHSDYMNMTPRRPGPTRKHYQPYAPPRDFAAYRSRVKFSRSADAPAYQQGQNQLYNELNLGRREEYDVLDKRRGRDPEMGGKPRRKNPQEGLYNELQKDKMAEAYSEIGMKGERRRGKGHDGLYQGLSTATKDTYDALHMQALPPR

SEQ ID NO: 8 - protein, 119 aa, Artificial sequence
  Anti-P329G-ds VH
EVKLLESGGGLVQPGGSLKLSCAASGFDFSRYWMNWVRQAPGKCLEWIGEITPDSSTINYTPSLKDKFIISRDNAKNTLYLQMIKVRSEDTALYYCVRPYDYGAWFASWGQGTLVTVSA

SEQ ID NO: 9 - protein, 109 aa, Artificial sequence
  Anti-P329G-ds VL
QAVVTQESALTTSPGETVTLTCRSSTGAVTTSNYANWVQEKPDHLFTGLIGGTNKRAPGVPARFSGSLIGDKAALTITGAQTEDEAIYFCALWYSNHWVFGCGTKLTVL

SEQ ID NO: 10 - protein, 248 aa, Artificial sequence
  Anti-P329G-ds-scFv
EVKLLESGGGLVQPGGSLKLSCAASGFDFSRYWMNWVRQAPGKCLEWIGEITPDSSTINYTPSLKDKFIISRDNAKNTLYLQMIKVRSEDTALYYCVRPYDYGAWFASWGQGTLVTVSAGGGGSGGGGSGGGGSGGGGSQAVVTQESALTTSPGETVTLTCRSSTGAVTTSNYANWVQEKPDHLFTGLIGGTNKRAPGVPARFSGSLIGDKAALTITGAQTEDEAIYFCALWYSNHWVFGCGTKLTVL

SEQ ID NO: 11 - protein, 27 aa, Artificial sequence
  CD28ATM
FWVLVVVGGVLACYSLLVTVAFIIFWV

SEQ ID NO: 12 - protein, 41 aa, Artificial sequence
  CD28CSD
RSKRSRLLHSDYMNMTPRRPGPTRKHYQPYAPPRDFAAYRS

SEQ ID NO: 13 - protein, 112 aa, Artificial sequence
  CD3zSSD
RVKFSRSADAPAYQQGQNQLYNELNLGRREEYDVLDKRRGRDPEMGGKPRRKNPQEGLYNELQKDKMAEAYSEIGMKGERRRGKGHDGLYQGLSTATKDTYDALHMQALPPR

SEQ ID NO: 14 - protein, 180 aa, Artificial sequence
  CD28ATM-CD28-CD3z
FWVLVVVGGVLACYSLLVTVAFIIFWVRSKRSRLLHSDYMNMTPRRPGPTRKHYQPYAPPRDFAAYRSRVKFSRSADAPAYQQGQNQLYNELNLGRREEYDVLDKRRGRDPEMGGKPRRKNPQEGLYNELQKDKMAEAYSEIGMKGERRRGKGHDGLYQGLSTATKDTYDALHMQALPPR

SEQ ID NO: 15 - protein, 238 aa, Artificial sequence
  eGFP
VSKGEELFTGVVPILVELDGDVNGHKFSVSGEGEGDATYGKLTLKFICTTGKLPVPWPTLVTTLTYGVQCFSRYPDHMKQHDFFKSAMPEGYVQERTIFFKDDGNYKTRAEVKFEGDTLVNRIELKGIDFKEDGNILGHKLEYNYNSHNVYIMADKQKNGIKVNFKIRHNIEDGSVQLADHYQQNTPIGDGPVLLPDNHYLSTQSALSKDPNEKRDHMVLLEFVTAAGITLGMDELYK

SEQ ID NO: 16 - protein, 20 aa, Artificial sequence
  (G4S)4 linker
GGGGSGGGGSGGGGSGGGGS

SEQ ID NO: 17 - protein, 5 aa, Artificial sequence
  G4S linker
GGGGS

SEQ ID NO: 18 - protein, 19 aa, Artificial sequence
  T2A linker
GEGRGSLLTCGDVEENPGP

SEQ ID NO: 19 - DNA, 1356 bp, Artificial sequence
  Anti-P329G-ds-scFv-CD28ATM-CD28CSD-CD3zSSD fusion pETR17096
atgggatggagctgtatcatcctcttcttggtagcaacagctaccggtgtgcattccgaggtgaagctgctggagagcggcggcggcctggtgcagcccggcggcagcctgaagctgagctgcgccgccagcggcttcgacttcagcaggtactggatgaactgggtgaggcaggcccccggcaagtgtctggagtggatcggcgagatcacccccgacagcagcaccatcaactacacccccagcctgaaggacaagttcatcatcagcagggacaacgccaagaacaccctgtacctgcagatgatcaaggtgaggagcgaggacaccgccctgtactactgcgtgaggccctacgactacggcgcctggttcgccagctggggccagggcaccctggtgaccgtgagcgccggagggggcggaagtggtggcgggggaagcggcgggggtggcagcggagggggcggatctcaggccgtggtgacccaggagagcgccctgaccaccagccccggcgagaccgtgaccctgacctgcaggagcagcaccggcgccgtgaccaccagcaactacgccaactgggtgcaggagaagcccgaccacctgttcaccggcctgatcggcggcaccaacaagagggcccccggcgtgcccgccaggttcagcggcagcctgatcggcgacaaggccgccctgaccatcaccggcgcccagaccgaggacgaggccatctacttctgcgccctgtggtacagcaaccactgggtgttcggctgtggcaccaagctgaccgtgctgggagggggcggatccttctgggtgctggtggtggtgggcggcgtgctggcctgctacagcctgctggtgaccgtggccttcatcatcttctgggtgaggagcaagaggagcaggctgctgcacagcgactacatgaacatgacccccaggaggcccggccccaccaggaagcactaccagccctacgccccccccagggacttcgccgcctacaggagcagggtgaagttcagcaggagcgccgacgcccccgcctaccagcagggccagaaccagctgtataacgagctgaacctgggcaggagggaggagtacgacgtgctggacaagaggaggggcagggaccccgagatgggcggcaagcccaggaggaagaacccccaggagggcctgtataacgagctgcagaaggacaagatggccgaggcctacagcgagatcggcatgaagggcgagaggaggaggggcaagggccacgacggcctgtaccagggcctgagcaccgccaccaaggacacctacgacgccctgcacatgcaggccctgccccccagg

SEQ ID NO: 20 - DNA, 357 bp, Artificial sequence
  Anti-P329G-ds VH
gaggtgaagctgctggagagcggcggcggcctggtgcagcccggcggcagcctgaagctgagctgcgccgccagcggcttcgacttcagcaggtactggatgaactgggtgaggcaggcccccggcaagtgtctggagtggatcggcgagatcacccccgacagcagcaccatcaactacacccccagcctgaaggacaagttcatcatcagcagggacaacgccaagaacaccctgtacctgcagatgatcaaggtgaggagcgaggacaccgccctgtactactgcgtgaggccctacgactacggcgcctggttcgccagctggggccagggcaccctggtgaccgtgagcgcc

SEQ ID NO: 21 - DNA, 327 bp, Artificial sequence
  Anti-P329G-ds VL
caggccgtggtgacccaggagagcgccctgaccaccagccccggcgagaccgtgaccctgacctgcaggagcagcaccggcgccgtgaccaccagcaactacgccaactgggtgcaggagaagcccgaccacctgttcaccggcctgatcggcggcaccaacaagagggcccccggcgtgcccgccaggttcagcggcagcctgatcggcgacaaggccgccctgaccatcaccggcgcccagaccgaggacgaggccatctacttctgcgccctgtggtacagcaaccactgggtgttcggctgtggcaccaagctgaccgtgctg

SEQ ID NO: 22 - DNA, 799 bp, Artificial sequence
  Anti-P329G-ds-scFv
atgggatggagctgtatcatcctcttcttggtagcaacagctaccggtgtgcattccgaggtgaagctgctggagagcggcggcggcctggtgcagcccggcggcagcctgaagctgagctgcgccgccagcggcttcgacttcagcaggtactggatgaactgggtgaggcaggcccccggcaagtgtctggagtggatcggcgagatcacccccgacagcagcaccatcaactacacccccagcctgaaggacaagttcatcatcagcagggacaacgccaagaacaccctgtacctgcagatgatcaaggtgaggagcgaggacaccgccctgtactactgcgtgaggccctacgactacggcgcctggttcgccagctggggccagggcaccctggtgaccgtgagcgccggagggggcggaagtggtggcgggggaagcggcgggggtggcagcggagggggcggatctcaggccgtggtgacccaggagagcgccctgaccaccagccccggcgagaccgtgaccctgacctgcaggagcagcaccggcgccgtgaccaccagcaactacgccaactgggtgcaggagaagcccgaccacctgttcaccggcctgatcggcggcaccaacaagagggcccccggcgtgcccgccaggttcagcggcagcctgatcggcgacaaggccgccctgaccatcaccggcgcccagaccgaggacgaggccatctacttctgcgccctgtggtacagcaaccactgggtgttcggctgtggcaccaagctgaccgtgc

SEQ ID NO: 23 - DNA, 647 bp, Artificial sequence
  IRES EV71, internal ribosomal entry side
cccgaagtaacttagaagctgtaaatcaacgatcaatagcaggtgtggcacaccagtcataccttgatcaagcacttctgtttccccggactgagtatcaataggctgctcgcgcggctgaaggagaaaacgttcgttacccgaccaactacttcgagaagcttagtaccaccatgaacgaggcagggtgtttcgctcagcacaaccccagtgtagatcaggctgatgagtcactgcaacccccatgggcgaccatggcagtggctgcgttggcggcctgcccatggagaaatccatgggacgctctaattctgacatggtgtgaagtgcctattgagctaactggtagtcctccggcccctgattgcggctaatcctaactgcggagcacatgctcacaaaccagtgggtggtgtgtcgtaacgggcaactctgcagcggaaccgactactttgggtgtccgtgtttccttttattcctatattggctgcttatggtgacaatcaaaaagttgttaccatatagctattggattggccatccggtgtgcaacagggcaactgtttacctatttattggttttgtaccattatcactgaagtctgtgatcactctcaaattcattttgaccctcaacacaatcaaac

SEQ ID NO: 24 - DNA, 81 bp, Artificial sequence
  CD28ATM
ttttgggtgctggtggtggttggtggagtcctggcttgctatagcttgctagtaacagtggcctttattattttctgggtg

SEQ ID NO: 25 - DNA, 123 bp, Artificial sequence
  CD28CSD
aggagtaagaggagcaggctcctgcacagtgactacatgaacatgactccccgccgccccgggcccacccgcaagcattaccagccctatgccccaccacgcgacttcgcagcctatcgctcc

SEQ ID NO: 26 - DNA, 336 bp, Artificial sequence
  CD3z SSD
agagtgaagttcagcaggagcgcagacgcccccgcgtaccagcagggccagaaccagctctataacgagctcaatctaggacgaagagaggagtacgatgttttggacaagagacgtggccgggaccctgagatggggggaaagccgagaaggaagaaccctcaggaaggcctgtacaatgaactgcagaaagataagatggcggaggcctacagtgagattgggatgaaaggcgagcgccggaggggcaaggggcacgatggcctttaccagggtctcagtacagccaccaaggacacctacgacgcccttcacatgcaggccctgccccctcgc

SEQ ID NO: 27 - DNA, 540 bp, Artificial sequence
  CD28ATM-CD28-CD3z
ttctgggtgctggtggtggtgggcggcgtgctggcctgctacagcctgctggtgaccgtggccttcatcatcttctgggtgaggagcaagaggagcaggctgctgcacagcgactacatgaacatgacccccaggaggcccggccccaccaggaagcactaccagccctacgccccccccagggacttcgccgcctacaggagcagggtgaagttcagcaggagcgccgacgcccccgcctaccagcagggccagaaccagctgtataacgagctgaacctgggcaggagggaggagtacgacgtgctggacaagaggaggggcagggaccccgagatgggcggcaagcccaggaggaagaacccccaggagggcctgtataacgagctgcagaaggacaagatggccgaggcctacagcgagatcggcatgaagggcgagaggaggaggggcaagggccacgacggcctgtaccagggcctgagcaccgccaccaaggacacctacgacgccctgcacatgcaggccctgccccccagg

SEQ ID NO: 28 - DNA, 63 bp, Artificial sequence
  T2A element
tccggagagggcagaggaagtcttctaacatgcggtgacgtggaggagaatcccggccctagg

SEQ ID NO: 29 - DNA, 717 bp, Artificial sequence
  eGFP
gtgagcaagggcgaggagctgttcaccggggtggtgcccatcctggtcgagctggacggcgacgtaaacggccacaagttcagcgtgtccggcgagggcgagggcgatgccacctacggcaagctgaccctgaagttcatctgcaccaccggcaagctgcccgtgccctggcccaccctcgtgaccaccctgacctacggcgtgcagtgcttcagccgctaccccgaccacatgaagcagcacgacttcttcaagtccgccatgcccgaaggctacgtccaggagcgcaccatcttcttcaaggacgacggcaactacaagacccgcgccgaggtgaagttcgagggcgacaccctggtgaaccgcatcgagctgaagggcatcgacttcaaggaggacggcaacatcctggggcacaagctggagtacaactacaacagccacaacgtctatatcatggccgacaagcagaagaacggcatcaaggtgaacttcaagatccgccacaacatcgaggacggcagcgtgcagctcgccgaccactaccagcagaacacccccatcggcgacggccccgtgctgctgcccgacaaccactacctgagcacccagtccgccctgagcaaagaccccaacgagaagcgcgatcacatggtcctgctggagttcgtgaccgccgccgggatcactctcggcatggacgagctgtacaagtga

SEQ ID NO: 30 - DNA, 2136 bp, Artificial sequence
  Anti-P329G-ds-scFv-CD28ATM-CD28CSD-CD3zSSD-eGFP fusion pETR17096
atgggatggagctgtatcatcctcttcttggtagcaacagctaccggtgtgcattccgaggtgaagctgctggagagcggcggcggcctggtgcagcccggcggcagcctgaagctgagctgcgccgccagcggcttcgacttcagcaggtactggatgaactgggtgaggcaggcccccggcaagtgtctggagtggatcggcgagatcacccccgacagcagcaccatcaactacacccccagcctgaaggacaagttcatcatcagcagggacaacgccaagaacaccctgtacctgcagatgatcaaggtgaggagcgaggacaccgccctgtactactgcgtgaggccctacgactacggcgcctggttcgccagctggggccagggcaccctggtgaccgtgagcgccggagggggcggaagtggtggcgggggaagcggcgggggtggcagcggagggggcggatctcaggccgtggtgacccaggagagcgccctgaccaccagccccggcgagaccgtgaccctgacctgcaggagcagcaccggcgccgtgaccaccagcaactacgccaactgggtgcaggagaagcccgaccacctgttcaccggcctgatcggcggcaccaacaagagggcccccggcgtgcccgccaggttcagcggcagcctgatcggcgacaaggccgccctgaccatcaccggcgcccagaccgaggacgaggccatctacttctgcgccctgtggtacagcaaccactgggtgttcggctgtggcaccaagctgaccgtgctgggagggggcggatccttctgggtgctggtggtggtgggcggcgtgctggcctgctacagcctgctggtgaccgtggccttcatcatcttctgggtgaggagcaagaggagcaggctgctgcacagcgactacatgaacatgacccccaggaggcccggccccaccaggaagcactaccagccctacgccccccccagggacttcgccgcctacaggagcagggtgaagttcagcaggagcgccgacgcccccgcctaccagcagggccagaaccagctgtataacgagctgaacctgggcaggagggaggagtacgacgtgctggacaagaggaggggcagggaccccgagatgggcggcaagcccaggaggaagaacccccaggagggcctgtataacgagctgcagaaggacaagatggccgaggcctacagcgagatcggcatgaagggcgagaggaggaggggcaagggccacgacggcctgtaccagggcctgagcaccgccaccaaggacacctacgacgccctgcacatgcaggccctgccccccaggtccggagagggcagaggaagtcttctaacatgcggtgacgtggaggagaatcccggccctagggtgagcaagggcgaggagctgttcaccggggtggtgcccatcctggtcgagctggacggcgacgtaaacggccacaagttcagcgtgtccggcgagggcgagggcgatgccacctacggcaagctgaccctgaagttcatctgcaccaccggcaagctgcccgtgccctggcccaccctcgtgaccaccctgacctacggcgtgcagtgcttcagccgctaccccgaccacatgaagcagcacgacttcttcaagtccgccatgcccgaaggctacgtccaggagcgcaccatcttcttcaaggacgacggcaactacaagacccgcgccgaggtgaagttcgagggcgacaccctggtgaaccgcatcgagctgaagggcatcgacttcaaggaggacggcaacatcctggggcacaagctggagtacaactacaacagccacaacgtctatatcatggccgacaagcagaagaacggcatcaaggtgaacttcaagatccgccacaacatcgaggacggcagcgtgcagctcgccgaccactaccagcagaacacccccatcggcgacggccccgtgctgctgcccgacaaccactacctgagcacccagtccgccctgagcaaagaccccaacgagaagcgcgatcacatggtcctgctggagttcgtgaccgccgccgggatcactctcggcatggacgagctgtacaagtga

SEQ ID NO: 31 - protein, 433 aa, Artificial sequence
  Anti-P329G-scFv- CD28ATM-CD28CSD-CD3zSSD fusion
EVKLLESGGGLVQPGGSLKLSCAASGFDFSRYWMNWVRQAPGKGLEWIGEITPDSSTINYTPSLKDKFIISRDNAKNTLYLQMIKVRSEDTALYYCVRPYDYGAWFASWGQGTLVTVSAGGGGSGGGGSGGGGSGGGGSQAVVTQESALTTSPGETVTLTCRSSTGAVTTSNYANWVQEKPDHLFTGLIGGTNKRAPGVPARFSGSLIGDKAALTITGAQTEDEAIYFCALWYSNHWVFGGGTKLTVLGGGGSFWVLVVVGGVLACYSLLVTVAFIIFWVRSKRSRLLHSDYMNMTPRRPGPTRKHYQPYAPPRDFAAYRSRVKFSRSADAPAYQQGQNQLYNELNLGRREEYDVLDKRRGRDPEMGGKPRRKNPQEGLYNELQKDKMAEAYSEIGMKGERRRGKGHDGLYQGLSTATKDTYDALHMQALPPR

SEQ ID NO: 32 - protein, 119 aa, Artificial sequence
  Anti-P329G VH
EVKLLESGGGLVQPGGSLKLSCAASGFDFSRYWMNWVRQAPGKGLEWIGEITPDSSTINYTPSLKDKFIISRDNAKNTLYLQMIKVRSEDTALYYCVRPYDYGAWFASWGQGTLVTVSA

SEQ ID NO: 33 - protein, 109 aa, Artificial sequence
  Anti-P329G VL
QAVVTQESALTTSPGETVTLTCRSSTGAVTTSNYANWVQEKPDHLFTGLIGGTNKRAPGVPARFSGSLIGDKAALTITGAQTEDEAIYFCALWYSNHWVFGGGTKLTVL

SEQ ID NO: 34 - protein, 248 aa, Artificial sequence
  Anti-P329G-scFv
EVKLLESGGGLVQPGGSLKLSCAASGFDFSRYWMNWVRQAPGKGLEWIGEITPDSSTINYTPSLKDKFIISRDNAKNTLYLQMIKVRSEDTALYYCVRPYDYGAWFASWGQGTLVTVSAGGGGSGGGGSGGGGSGGGGSQAVVTQESALTTSPGETVTLTCRSSTGAVTTSNYANWVQEKPDHLFTGLIGGTNKRAPGVPARFSGSLIGDKAALTITGAQTEDEAIYFCALWYSNHWVFGGGTKLTVL

SEQ ID NO: 35 - DNA, 1356 bp, Artificial sequence
  Anti-P329G-scFv-CD28ATM-CD28CSD-CD3zSSD fusion
atgggatggagctgtatcatcctcttcttggtagcaacagctaccggtgtgcattccgaggtgaagctgctggagagcggcggcggcctggtgcagcccggcggcagcctgaagctgagctgcgccgccagcggcttcgacttcagcaggtactggatgaactgggtgaggcaggcccccggcaagggtctggagtggatcggcgagatcacccccgacagcagcaccatcaactacacccccagcctgaaggacaagttcatcatcagcagggacaacgccaagaacaccctgtacctgcagatgatcaaggtgaggagcgaggacaccgccctgtactactgcgtgaggccctacgactacggcgcctggttcgccagctggggccagggcaccctggtgaccgtgagcgccggagggggcggaagtggtggcgggggaagcggcgggggtggcagcggagggggcggatctcaggccgtggtgacccaggagagcgccctgaccaccagccccggcgagaccgtgaccctgacctgcaggagcagcaccggcgccgtgaccaccagcaactacgccaactgggtgcaggagaagcccgaccacctgttcaccggcctgatcggcggcaccaacaagagggcccccggcgtgcccgccaggttcagcggcagcctgatcggcgacaaggccgccctgaccatcaccggcgcccagaccgaggacgaggccatctacttctgcgccctgtggtacagcaaccactgggtgttcggcggtggcaccaagctgaccgtgctgggagggggcggatccttctgggtgctggtggtggtgggcggcgtgctggcctgctacagcctgctggtgaccgtggccttcatcatcttctgggtgaggagcaagaggagcaggctgctgcacagcgactacatgaacatgacccccaggaggcccggccccaccaggaagcactaccagccctacgccccccccagggacttcgccgcctacaggagcagggtgaagttcagcaggagcgccgacgcccccgcctaccagcagggccagaaccagctgtataacgagctgaacctgggcaggagggaggagtacgacgtgctggacaagaggaggggcagggaccccgagatgggcggcaagcccaggaggaagaacccccaggagggcctgtataacgagctgcagaaggacaagatggccgaggcctacagcgagatcggcatgaagggcgagaggaggaggggcaagggccacgacggcctgtaccagggcctgagcaccgccaccaaggacacctacgacgccctgcacatgcaggccctgccccccagg

SEQ ID NO: 36 - DNA, 357 bp, Artificial sequence
  Anti-P329G VH
gaggtgaagctgctggagagcggcggcggcctggtgcagcccggcggcagcctgaagctgagctgcgccgccagcggcttcgacttcagcaggtactggatgaactgggtgaggcaggcccccggcaagggtctggagtggatcggcgagatcacccccgacagcagcaccatcaactacacccccagcctgaaggacaagttcatcatcagcagggacaacgccaagaacaccctgtacctgcagatgatcaaggtgaggagcgaggacaccgccctgtactactgcgtgaggccctacgactacggcgcctggttcgccagctggggccagggcaccctggtgaccgtgagcgcc

SEQ ID NO: 37 - DNA, 327 bp, Artificial sequence
  Anti-P329G VL
caggccgtggtgacccaggagagcgccctgaccaccagccccggcgagaccgtgaccctgacctgcaggagcagcaccggcgccgtgaccaccagcaactacgccaactgggtgcaggagaagcccgaccacctgttcaccggcctgatcggcggcaccaacaagagggcccccggcgtgcccgccaggttcagcggcagcctgatcggcgacaaggccgccctgaccatcaccggcgcccagaccgaggacgaggccatctacttctgcgccctgtggtacagcaaccactgggtgttcggcggtggcaccaagctgaccgtgctg

SEQ ID NO: 38 - DNA, 2136 bp, Artificial sequence
  Anti-P329G-scFv-CD28ATM-CD28CSD-CD3zSSD-eGFP fusion
atgggatggagctgtatcatcctcttcttggtagcaacagctaccggtgtgcattccgaggtgaagctgctggagagcggcggcggcctggtgcagcccggcggcagcctgaagctgagctgcgccgccagcggcttcgacttcagcaggtactggatgaactgggtgaggcaggcccccggcaagggtctggagtggatcggcgagatcacccccgacagcagcaccatcaactacacccccagcctgaaggacaagttcatcatcagcagggacaacgccaagaacaccctgtacctgcagatgatcaaggtgaggagcgaggacaccgccctgtactactgcgtgaggccctacgactacggcgcctggttcgccagctggggccagggcaccctggtgaccgtgagcgccggagggggcggaagtggtggcgggggaagcggcgggggtggcagcggagggggcggatctcaggccgtggtgacccaggagagcgccctgaccaccagccccggcgagaccgtgaccctgacctgcaggagcagcaccggcgccgtgaccaccagcaactacgccaactgggtgcaggagaagcccgaccacctgttcaccggcctgatcggcggcaccaacaagagggcccccggcgtgcccgccaggttcagcggcagcctgatcggcgacaaggccgccctgaccatcaccggcgcccagaccgaggacgaggccatctacttctgcgccctgtggtacagcaaccactgggtgttcggcggtggcaccaagctgaccgtgctgggagggggcggatccttctgggtgctggtggtggtgggcggcgtgctggcctgctacagcctgctggtgaccgtggccttcatcatcttctgggtgaggagcaagaggagcaggctgctgcacagcgactacatgaacatgacccccaggaggcccggccccaccaggaagcactaccagccctacgccccccccagggacttcgccgcctacaggagcagggtgaagttcagcaggagcgccgacgcccccgcctaccagcagggccagaaccagctgtataacgagctgaacctgggcaggagggaggagtacgacgtgctggacaagaggaggggcagggaccccgagatgggcggcaagcccaggaggaagaacccccaggagggcctgtataacgagctgcagaaggacaagatggccgaggcctacagcgagatcggcatgaagggcgagaggaggaggggcaagggccacgacggcctgtaccagggcctgagcaccgccaccaaggacacctacgacgccctgcacatgcaggccctgccccccaggtccggagagggcagaggaagtcttctaacatgcggtgacgtggaggagaatcccggccctagggtgagcaagggcgaggagctgttcaccggggtggtgcccatcctggtcgagctggacggcgacgtaaacggccacaagttcagcgtgtccggcgagggcgagggcgatgccacctacggcaagctgaccctgaagttcatctgcaccaccggcaagctgcccgtgccctggcccaccctcgtgaccaccctgacctacggcgtgcagtgcttcagccgctaccccgaccacatgaagcagcacgacttcttcaagtccgccatgcccgaaggctacgtccaggagcgcaccatcttcttcaaggacgacggcaactacaagacccgcgccgaggtgaagttcgagggcgacaccctggtgaaccgcatcgagctgaagggcatcgacttcaaggaggacggcaacatcctggggcacaagctggagtacaactacaacagccacaacgtctatatcatggccgacaagcagaagaacggcatcaaggtgaacttcaagatccgccacaacatcgaggacggcagcgtgcagctcgccgaccactaccagcagaacacccccatcggcgacggccccgtgctgctgcccgacaaccactacctgagcacccagtccgccctgagcaaagaccccaacgagaagcgcgatcacatggtcctgctggagttcgtgaccgccgccgggatcactctcggcatggacgagctgtacaagtga

SEQ ID NO: 39 - protein, 407 aa, Artificial sequence
  Anti-P329G-ds-Fab- heavy chain-CD28ATM-CD28CSD-CD3zSSD fusion pETR17100
EVKLLESGGGLVQPGGSLKLSCAASGFDFSRYWMNWVRQAPGKCLEWIGEITPDSSTINYTPSLKDKFIISRDNAKNTLYLQMIKVRSEDTALYYCVRPYDYGAWFASWGQGTLVTVSAASTKGPSVFPLAPSSKSTSGGTAALGCLVKDYFPEPVTVSWNSGALTSGVHTFPAVLQSSGLYSLSSVVTVPSSSLGTQTYICNVNHKPSNTKVDKKVEPKSCGGGGSFWVLVVVGGVLACYSLLVTVAFIIFWVRSKRSRLLHSDYMNMTPRRPGPTRKHYQPYAPPRDFAAYRSRVKFSRSADAPAYQQGQNQLYNELNLGRREEYDVLDKRRGRDPEMGGKPRRKNPQEGLYNELQKDKMAEAYSEIGMKGERRRGKGHDGLYQGLSTATKDTYDALHMQALPPR

SEQ ID NO: 40 - protein, 222 aa, Artificial sequence
  Anti-P329G-ds-Fab heavy chain
EVKLLESGGGLVQPGGSLKLSCAASGFDFSRYWMNWVRQAPGKCLEWIGEITPDSSTINYTPSLKDKFIISRDNAKNTLYLQMIKVRSEDTALYYCVRPYDYGAWFASWGQGTLVTVSAASTKGPSVFPLAPSSKSTSGGTAALGCLVKDYFPEPVTVSWNSGALTSGVHTFPAVLQSSGLYSLSSVVTVPSSSLGTQTYICNVNHKPSNTKVDKKVEPKSC

SEQ ID NO: 41 - protein, 216 aa, Artificial sequence
  Anti P329G-ds-Fab light chain
QAVVTQESALTTSPGETVTLTCRSSTGAVTTSNYANWVQEKPDHLFTGLIGGTNKRAPGVPARFSGSLIGDKAALTITGAQTEDEAIYFCALWYSNHWVFGCGTKLTVLRTVAAPSVFIFPPSDEQLKSGTASVVCLLNNFYPREAKVQWKVDNALQSGNSQESVTEQDSKDSTYSLSSTLTLSKADYEKHKVYACEVTHQGLSSPVTKSFNRGEC

SEQ ID NO: 42 - protein, 107 aa, Artificial sequence [sequence omitted]

SEQ ID NO: 43 - protein, 103 aa, Artificial sequence
  CH1
ASTKGPSVFPLAPSSKSTSGGTAALGCLVKDYFPEPVTVSWNSGALTSGVHTFPAVLQSSGLYSLSSVVTVPSSSLGTQTYICNVNHKPSNTKVDKKVEPKSC

SEQ ID NO: 44 - DNA, 2645 bp, Artificial sequence
  Anti-P329G-ds-Fab-heavy chain-CD28ATM-CD28CSD-CD3zSSD fusion pETR17100
atgggatggagctgtatcatcctcttcttggtagcaacagctacgggtgtgcattcccaggccgtggtgacccaggagagcgccctgaccaccagccccggcgagaccgtgaccctgacctgcaggagcagcaccggcgccgtgaccaccagcaactacgccaactgggtgcaggagaagcccgaccacctgttcaccggcctgatcggcggcaccaacaagagggcccccggcgtgcccgccaggttcagcggcagcctgatcggcgacaaggccgccctgaccatcaccggcgcccagaccgaggacgaggccatctacttctgcgccctgtggtacagcaaccactgggtgttcggctgtggcaccaagctgaccgtgctgcgtacggtggctgcaccatctgtcttcatcttcccgccatctgatgagcagttgaaatctggaactgcctctgttgtgtgcctgctgaataacttctatcccagagaggccaaagtacagtggaaggtggataacgccctccaatcgggtaactcccaggagagtgtcacagagcaggacagcaaggacagcacctacagcctcagcagcaccctgacgctgagcaaagcagactacgagaaacacaaagtctacgcctgcgaagtcacccatcagggcctgagctcgcccgtcacaaagagcttcaacaggggagagtgttaggaattccccgaagtaacttagaagctgtaaatcaacgatcaatagcaggtgtggcacaccagtcataccttgatcaagcacttctgtttccccggactgagtatcaataggctgctcgcgcggctgaaggagaaaacgttcgttacccgaccaactacttcgagaagcttagtaccaccatgaacgaggcagggtgtttcgctcagcacaaccccagtgtagatcaggctgatgagtcactgcaacccccatgggcgaccatggcagtggctgcgttggcggcctgcccatggagaaatccatgggacgctctaattctgacatggtgtgaagtgcctattgagctaactggtagtcctccggcccctgattgcggctaatcctaactgcggagcacatgctcacaaaccagtgggtggtgtgtcgtaacgggcaactctgcagcggaaccgactactttgggtgtccgtgtttccttttattcctatattggctgcttatggtgacaatcaaaaagttgttaccatatagctattggattggccatccggtgtgcaacagggcaactgtttacctatttattggttttgtaccattatcactgaagtctgtgatcactctcaaattcattttgaccctcaacacaatcaaacgccaccatgggatggagctgtatcatcctcttcttggtagcaacagctaccggtgtgcactccgaggtgaagctgctggagagcggcggcggcctggtgcagcccggcggcagcctgaagctgagctgcgccgccagcggcttcgacttcagcaggtactggatgaactgggtgaggcaggcccccggcaagtgtctggagtggatcggcgagatcacccccgacagcagcaccatcaactacacccccagcctgaaggacaagttcatcatcagcagggacaacgccaagaacaccctgtacctgcagatgatcaaggtgaggagcgaggacaccgccctgtactactgcgtgaggccctacgactacggcgcctggttcgccagctggggccagggcaccctggtgaccgtgagcgccgctagcaccaagggcccctccgtgttccccctggcccccagcagcaagagcaccagcggcggcacagccgctctgggctgcctggtcaaggactacttccccgagcccgtgaccgtgtcctggaacagcggagccctgacctccggcgtgcacaccttccccgccgtgctgcagagttctggcctgtatagcctgagcagcgtggtcaccgtgccttctagcagcctgggcacccagacctacatctgcaacgtgaaccacaagcccagcaacaccaaggtggacaagaaggtggagcccaagagctgcggagggggcggatccttctgggtgctggtggtggtgggcggcgtgctggcctgctacagcctgctggtgaccgtggccttcatcatcttctgggtgaggagcaagaggagcaggctgctgcacagcgactacatgaacatgacccccaggaggcccggccccaccaggaagcactaccagccctacgccccccccagggacttcgccgcctacaggagcagggtgaagttcagcaggagcgccgacgcccccgcctaccagcagggccagaaccagctgtataacgagctgaacctgggcaggagggaggagtacgacgtgctggacaagaggaggggcagggaccccgagatgggcggcaagcccaggaggaagaacccccaggagggcctgtataacgagctgcagaaggacaagatggccgaggcctacagcgagatcggcatgaagggcgagaggaggaggggcaagggccacgacggcctgtaccagggcctgagcaccgccaccaaggacacctacgacgccctgcacatgcaggccctgccccccagg

SEQ ID NO: 45 - DNA, 324 bp, Artificial sequence
  CL
cgtacggtggctgcaccatctgtcttcatcttcccgccatctgatgagcagttgaaatctggaactgcctctgttgtgtgcctgctgaataacttctatcccagagaggccaaagtacagtggaaggtggataacgccctccaatcgggtaactcccaggagagtgtcacagagcaggacagcaaggacagcacctacagcctcagcagcaccctgacgctgagcaaagcagactacgagaaacacaaagtctacgcctgcgaagtcacccatcagggcctgagctcgcccgtcacaaagagcttcaacaggggagagtgttag

SEQ ID NO: 46 - DNA, 309 bp, Artificial sequence
  CH1
gctagcaccaagggcccctccgtgttccccctggcccccagcagcaagagcaccagcggcggcacagccgctctgggctgcctggtcaaggactacttccccgagcccgtgaccgtgtcctggaacagcggagccctgacctccggcgtgcacaccttccccgccgtgctgcagagttctggcctgtatagcctgagcagcgtggtcaccgtgccttctagcagcctgggcacccagacctacatctgcaacgtgaaccacaagcccagcaacaccaaggtggacaagaaggtggagcccaagagctgc

SEQ ID NO: 47 - DNA, 3425 bp, Artificial sequence
  Anti-P329G-ds-Fab-heavy chain-CD28TM-CD28CSD-CD3ZSSD-eGFP fusion pETR17100
atgggatggagctgtatcatcctcttcttggtagcaacagctacgggtgtgcattcccaggccgtggtgacccaggagagcgccctgaccaccagccccggcgagaccgtgaccctgacctgcaggagcagcaccggcgccgtgaccaccagcaactacgccaactgggtgcaggagaagcccgaccacctgttcaccggcctgatcggcggcaccaacaagagggcccccggcgtgcccgccaggttcagcggcagcctgatcggcgacaaggccgccctgaccatcaccggcgcccagaccgaggacgaggccatctacttctgcgccctgtggtacagcaaccactgggtgttcggctgtggcaccaagctgaccgtgctgcgtacggtggctgcaccatctgtcttcatcttcccgccatctgatgagcagttgaaatctggaactgcctctgttgtgtgcctgctgaataacttctatcccagagaggccaaagtacagtggaaggtggataacgccctccaatcgggtaactcccaggagagtgtcacagagcaggacagcaaggacagcacctacagcctcagcagcaccctgacgctgagcaaagcagactacgagaaacacaaagtctacgcctgcgaagtcacccatcagggcctgagctcgcccgtcacaaagagcttcaacaggggagagtgttaggaattccccgaagtaacttagaagctgtaaatcaacgatcaatagcaggtgtggcacaccagtcataccttgatcaagcacttctgtttccccggactgagtatcaataggctgctcgcgcggctgaaggagaaaacgttcgttacccgaccaactacttcgagaagcttagtaccaccatgaacgaggcagggtgtttcgctcagcacaaccccagtgtagatcaggctgatgagtcactgcaacccccatgggcgaccatggcagtggctgcgttggcggcctgcccatggagaaatccatgggacgctctaattctgacatggtgtgaagtgcctattgagctaactggtagtcctccggcccctgattgcggctaatcctaactgcggagcacatgctcacaaaccagtgggtggtgtgtcgtaacgggcaactctgcagcggaaccgactactttgggtgtccgtgtttccttttattcctatattggctgcttatggtgacaatcaaaaagttgttaccatatagctattggattggccatccggtgtgcaacagggcaactgtttacctatttattggttttgtaccattatcactgaagtctgtgatcactctcaaattcattttgaccctcaacacaatcaaacgccaccatgggatggagctgtatcatcctcttcttggtagcaacagctaccggtgtgcactccgaggtgaagctgctggagagcggcggcggcctggtgcagcccggcggcagcctgaagctgagctgcgccgccagcggcttcgacttcagcaggtactggatgaactgggtgaggcaggcccccggcaagtgtctggagtggatcggcgagatcacccccgacagcagcaccatcaactacacccccagcctgaaggacaagttcatcatcagcagggacaacgccaagaacaccctgtacctgcagatgatcaaggtgaggagcgaggacaccgccctgtactactgcgtgaggccctacgactacggcgcctggttcgccagctggggccagggcaccctggtgaccgtgagcgccgctagcaccaagggcccctccgtgttccccctggcccccagcagcaagagcaccagcggcggcacagccgctctgggctgcctggtcaaggactacttccccgagcccgtgaccgtgtcctggaacagcggagccctgacctccggcgtgcacaccttccccgccgtgctgcagagttctggcctgtatagcctgagcagcgtggtcaccgtgccttctagcagcctgggcacccagacctacatctgcaacgtgaaccacaagcccagcaacaccaaggtggacaagaaggtggagcccaagagctgcggagggggcggatccttctgggtgctggtggtggtgggcggcgtgctggcctgctacagcctgctggtgaccgtggccttcatcatcttctgggtgaggagcaagaggagcaggctgctgcacagcgactacatgaacatgacccccaggaggcccggccccaccaggaagcactaccagccctacgccccccccagggacttcgccgcctacaggagcagggtgaagttcagcaggagcgccgacgcccccgcctaccagcagggccagaaccagctgtataacgagctgaacctgggcaggagggaggagtacgacgtgctggacaagaggaggggcagggaccccgagatgggcggcaagcccaggaggaagaacccccaggagggcctgtataacgagctgcagaaggacaagatggccgaggcctacagcgagatcggcatgaagggcgagaggaggaggggcaagggccacgacggcctgtaccagggcctgagcaccgccaccaaggacacctacgacgccctgcacatgcaggccctgccccccaggtccggagagggcagaggaagtcttctaacatgcggtgacgtggaggagaatcccggccctagggtgagcaagggcgaggagctgttcaccggggtggtgcccatcctggtcgagctggacggcgacgtaaacggccacaagttcagcgtgtccggcgagggcgagggcgatgccacctacggcaagctgaccctgaagttcatctgcaccaccggcaagctgcccgtgccctggcccaccctcgtgaccaccctgacctacggcgtgcagtgcttcagccgctaccccgaccacatgaagcagcacgacttcttcaagtccgccatgcccgaaggctacgtccaggagcgcaccatcttcttcaaggacgacggcaactacaagacccgcgccgaggtgaagttcgagggcgacaccctggtgaaccgcatcgagctgaagggcatcgacttcaaggaggacggcaacatcctggggcacaagctggagtacaactacaacagccacaacgtctatatcatggccgacaagcagaagaacggcatcaaggtgaacttcaagatccgccacaacatcgaggacggcagcgtgcagctcgccgaccactaccagcagaacacccccatcggcgacggccccgtgctgctgcccgacaaccactacctgagcacccagtccgccctgagcaaagaccccaacgagaagcgcgatcacatggtcctgctggagttcgtgaccgccgccgggatcactctcggcatggacgagctgtacaagtga

SEQ ID NO: 48 - protein, 407 aa, Artificial sequence
  Anti-P329G-Fab-heavy chain-CD28ATM-CD28CSD-CD3zSSD fusion pETR17594
EVKLLESGGGLVQPGGSLKLSCAASGFDFSRYWMNWVRQAPGKGLEWIGEITPDSSTINYTPSLKDKFIISRDNAKNTLYLQMIKVRSEDTALYYCVRPYDYGAWFASWGQGTLVTVSAASTKGPSVFPLAPSSKSTSGGTAALGCLVKDYFPEPVTVSWNSGALTSGVHTFPAVLQSSGLYSLSSVVTVPSSSLGTQTYICNVNHKPSNTKVDKKVEPKSCGGGGSFWVLVVVGGVLACYSLLVTVAFIIFWVRSKRSRLLHSDYMNMTPRRPGPTRKHYQPYAPPRDFAAYRSRVKFSRSADAPAYQQGQNQLYNELNLGRREEYDVLDKRRGRDPEMGGKPRRKNPQEGLYNELQKDKMAEAYSEIGMKGERRRGKGHDGLYQGLSTATKDTYDALHMQALPPR

SEQ ID NO: 49 - protein, 222 aa, Artificial sequence
  Anti-P329G-Fab heavy chain
EVKLLESGGGLVQPGGSLKLSCAASGFDFSRYWMNWVRQAPGKGLEWIGEITPDSSTINYTPSLKDKFIISRDNAKNTLYLQMIKVRSEDTALYYCVRPYDYGAWFASWGQGTLVTVSAASTKGPSVFPLAPSSKSTSGGTAALGCLVKDYFPEPVTVSWNSGALTSGVHTFPAVLQSSGLYSLSSVVTVPSSSLGTQTYICNVNHKPSNTKVDKKVEPKSC

SEQ ID NO: 50 - protein, 216 aa, Artificial sequence
  Anti-P329G-Fab light chain
QAVVTQESALTTSPGETVTLTCRSSTGAVTTSNYANWVQEKPDHLFTGLIGGTNKRAPGVPARFSGSLIGDKAALTITGAQTEDEAIYFCALWYSNHWVFGGGTKLTVLRTVAAPSVFIFPPSDEQLKSGTASVVCLLNNFYPREAKVQWKVDNALQSGNSQESVTEQDSKDSTYSLSSTLTLSKADYEKHKVYACEVTHQGLSSPVTKSFNRGEC

SEQ ID NO: 51 - DNA, 2645 bp, Artificial sequence
  Anti-P329G-Fab-heavy chain-CD28ATM-CD28CSD-CD3zSSD fusion pETR17594
atgggatggagctgtatcatcctcttcttggtagcaacagctacgggtgtgcattcccaggccgtggtgacccaggagagcgccctgaccaccagccccggcgagaccgtgaccctgacctgcaggagcagcaccggcgccgtgaccaccagcaactacgccaactgggtgcaggagaagcccgaccacctgttcaccggcctgatcggcggcaccaacaagagggcccccggcgtgcccgccaggttcagcggcagcctgatcggcgacaaggccgccctgaccatcaccggcgcccagaccgaggacgaggccatctacttctgcgccctgtggtacagcaaccactgggtgttcggcggtggcaccaagctgaccgtgctgcgtacggtggctgcaccatctgtcttcatcttcccgccatctgatgagcagttgaaatctggaactgcctctgttgtgtgcctgctgaataacttctatcccagagaggccaaagtacagtggaaggtggataacgccctccaatcgggtaactcccaggagagtgtcacagagcaggacagcaaggacagcacctacagcctcagcagcaccctgacgctgagcaaagcagactacgagaaacacaaagtctacgcctgcgaagtcacccatcagggcctgagctcgcccgtcacaaagagcttcaacaggggagagtgttaggaattccccgaagtaacttagaagctgtaaatcaacgatcaatagcaggtgtggcacaccagtcataccttgatcaagcacttctgtttccccggactgagtatcaataggctgctcgcgcggctgaaggagaaaacgttcgttacccgaccaactacttcgagaagcttagtaccaccatgaacgaggcagggtgtttcgctcagcacaaccccagtgtagatcaggctgatgagtcactgcaacccccatgggcgaccatggcagtggctgcgttggcggcctgcccatggagaaatccatgggacgctctaattctgacatggtgtgaagtgcctattgagctaactggtagtcctccggcccctgattgcggctaatcctaactgcggagcacatgctcacaaaccagtgggtggtgtgtcgtaacgggcaactctgcagcggaaccgactactttgggtgtccgtgtttccttttattcctatattggctgcttatggtgacaatcaaaaagttgttaccatatagctattggattggccatccggtgtgcaacagggcaactgtttacctatttattggttttgtaccattatcactgaagtctgtgatcactctcaaattcattttgaccctcaacacaatcaaacgccaccatgggatggagctgtatcatcctcttcttggtagcaacagctaccggtgtgcactccgaggtgaagctgctggagagcggcggcggcctggtgcagcccggcggcagcctgaagctgagctgcgccgccagcggcttcgacttcagcaggtactggatgaactgggtgaggcaggcccccggcaagggtctggagtggatcggcgagatcacccccgacagcagcaccatcaactacacccccagcctgaaggacaagttcatcatcagcagggacaacgccaagaacaccctgtacctgcagatgatcaaggtgaggagcgaggacaccgccctgtactactgcgtgaggccctacgactacggcgcctggttcgccagctggggccagggcaccctggtgaccgtgagcgccgctagcaccaagggcccctccgtgttccccctggcccccagcagcaagagcaccagcggcggcacagccgctctgggctgcctggtcaaggactacttccccgagcccgtgaccgtgtcctggaacagcggagccctgacctccggcgtgcacaccttccccgccgtgctgcagagttctggcctgtatagcctgagcagcgtggtcaccgtgccttctagcagcctgggcacccagacctacatctgcaacgtgaaccacaagcccagcaacaccaaggtggacaagaaggtggagcccaagagctgcggagggggcggatccttctgggtgctggtggtggtgggcggcgtgctggcctgctacagcctgctggtgaccgtggccttcatcatcttctgggtgaggagcaagaggagcaggctgctgcacagcgactacatgaacatgacccccaggaggcccggccccaccaggaagcactaccagccctacgccccccccagggacttcgccgcctacaggagcagggtgaagttcagcaggagcgccgacgcccccgcctaccagcagggccagaaccagctgtataacgagctgaacctgggcaggagggaggagtacgacgtgctggacaagaggaggggcagggaccccgagatgggcggcaagcccaggaggaagaacccccaggagggcctgtataacgagctgcagaaggacaagatggccgaggcctacagcgagatcggcatgaagggcgagaggaggaggggcaagggccacgacggcctgtaccagggcctgagcaccgccaccaaggacacctacgacgccctgcacatgcaggccctgccccccagg

SEQ ID NO: 52 - DNA, 3425 bp, Artificial sequence
  Anti-P329G-Fab-heavy chain-CD28ATM-CD28CSD-CD3zSSD-eGFP fusion pETR17594
atgggatggagctgtatcatcctcttcttggtagcaacagctacgggtgtgcattcccaggccgtggtgacccaggagagcgccctgaccaccagccccggcgagaccgtgaccctgacctgcaggagcagcaccggcgccgtgaccaccagcaactacgccaactgggtgcaggagaagcccgaccacctgttcaccggcctgatcggcggcaccaacaagagggcccccggcgtgcccgccaggttcagcggcagcctgatcggcgacaaggccgccctgaccatcaccggcgcccagaccgaggacgaggccatctacttctgcgccctgtggtacagcaaccactgggtgttcggcggtggcaccaagctgaccgtgctgcgtacggtggctgcaccatctgtcttcatcttcccgccatctgatgagcagttgaaatctggaactgcctctgttgtgtgcctgctgaataacttctatcccagagaggccaaagtacagtggaaggtggataacgccctccaatcgggtaactcccaggagagtgtcacagagcaggacagcaaggacagcacctacagcctcagcagcaccctgacgctgagcaaagcagactacgagaaacacaaagtctacgcctgcgaagtcacccatcagggcctgagctcgcccgtcacaaagagcttcaacaggggagagtgttaggaattccccgaagtaacttagaagctgtaaatcaacgatcaatagcaggtgtggcacaccagtcataccttgatcaagcacttctgtttccccggactgagtatcaataggctgctcgcgcggctgaaggagaaaacgttcgttacccgaccaactacttcgagaagcttagtaccaccatgaacgaggcagggtgtttcgctcagcacaaccccagtgtagatcaggctgatgagtcactgcaacccccatgggcgaccatggcagtggctgcgttggcggcctgcccatggagaaatccatgggacgctctaattctgacatggtgtgaagtgcctattgagctaactggtagtcctccggcccctgattgcggctaatcctaactgcggagcacatgctcacaaaccagtgggtggtgtgtcgtaacgggcaactctgcagcggaaccgactactttgggtgtccgtgtttccttttattcctatattggctgcttatggtgacaatcaaaaagttgttaccatatagctattggattggccatccggtgtgcaacagggcaactgtttacctatttattggttttgtaccattatcactgaagtctgtgatcactctcaaattcattttgaccctcaacacaatcaaacgccaccatgggatggagctgtatcatcctcttcttggtagcaacagctaccggtgtgcactccgaggtgaagctgctggagagcggcggcggcctggtgcagcccggcggcagcctgaagctgagctgcgccgccagcggcttcgacttcagcaggtactggatgaactgggtgaggcaggcccccggcaagggtctggagtggatcggcgagatcacccccgacagcagcaccatcaactacacccccagcctgaaggacaagttcatcatcagcagggacaacgccaagaacaccctgtacctgcagatgatcaaggtgaggagcgaggacaccgccctgtactactgcgtgaggccctacgactacggcgcctggttcgccagctggggccagggcaccctggtgaccgtgagcgccgctagcaccaagggcccctccgtgttccccctggcccccagcagcaagagcaccagcggcggcacagccgctctgggctgcctggtcaaggactacttccccgagcccgtgaccgtgtcctggaacagcggagccctgacctccggcgtgcacaccttccccgccgtgctgcagagttctggcctgtatagcctgagcagcgtggtcaccgtgccttctagcagcctgggcacccagacctacatctgcaacgtgaaccacaagcccagcaacaccaaggtggacaagaaggtggagcccaagagctgcggagggggcggatccttctgggtgctggtggtggtgggcggcgtgctggcctgctacagcctgctggtgaccgtggccttcatcatcttctgggtgaggagcaagaggagcaggctgctgcacagcgactacatgaacatgacccccaggaggcccggccccaccaggaagcactaccagccctacgccccccccagggacttcgccgcctacaggagcagggtgaagttcagcaggagcgccgacgcccccgcctaccagcagggccagaaccagctgtataacgagctgaacctgggcaggagggaggagtacgacgtgctggacaagaggaggggcagggaccccgagatgggcggcaagcccaggaggaagaacccccaggagggcctgtataacgagctgcagaaggacaagatggccgaggcctacagcgagatcggcatgaagggcgagaggaggaggggcaagggccacgacggcctgtaccagggcctgagcaccgccaccaaggacacctacgacgccctgcacatgcaggccctgccccccaggtccggagagggcagaggaagtcttctaacatgcggtgacgtggaggagaatcccggccctagggtgagcaagggcgaggagctgttcaccggggtggtgcccatcctggtcgagctggacggcgacgtaaacggccacaagttcagcgtgtccggcgagggcgagggcgatgccacctacggcaagctgaccctgaagttcatctgcaccaccggcaagctgcccgtgccctggcccaccctcgtgaccaccctgacctacggcgtgcagtgcttcagccgctaccccgaccacatgaagcagcacgacttcttcaagtccgccatgcccgaaggctacgtccaggagcgcaccatcttcttcaaggacgacggcaactacaagacccgcgccgaggtgaagttcgagggcgacaccctggtgaaccgcatcgagctgaagggcatcgacttcaaggaggacggcaacatcctggggcacaagctggagtacaactacaacagccacaacgtctatatcatggccgacaagcagaagaacggcatcaaggtgaacttcaagatccgccacaacatcgaggacggcagcgtgcagctcgccgaccactaccagcagaacacccccatcggcgacggccccgtgctgctgcccgacaaccactacctgagcacccagtccgccctgagcaaagaccccaacgagaagcgcgatcacatggtcctgctggagttcgtgaccgccgccgggatcactctcggcatggacgagctgtacaagtga

SEQ ID NO: 53 - protein, 5 aa, Artificial sequence
  Anti-AAA CDR H1 Kabat
SYGMS

SEQ ID NO: 54 - protein, 6 aa, Artificial sequence
  Anti-AAA CDR H2 Kabat
SSGGSY

SEQ ID NO: 55 - protein, 12 aa, Artificial sequence
  Anti-AAA CDR H3 Kabat
LGMITTGYAMDY

SEQ ID NO: 56 - protein, 16 aa, Artificial sequence
  Anti-AAA CDR L1 Kabat
RSSQTIVHSTGHTYLE

SEQ ID NO: 57 - protein, 7 aa, Artificial sequence
  Anti-AAA CDR L2 Kabat
KVSNRFS

SEQ ID NO: 58 - protein, 9 aa, Artificial sequence
  Anti-AAA CDR L3 Kabat
FQGSHVPYT

SEQ ID NO: 59 - protein, 457 aa, Artificial sequence
  Anti-AAA-scFv-CD28ATM-CD28CSD-CD3zSSD fusion
MNFGLSLVFLALILKGVQCEVQLVESGGDLVKPGGSLKLSCAASGFTFSSYGMSWVRQTPDKRLEWVATISSGGSYIYYPDSVKGRFTISRDNAKNTLYLQMSSLKSEDTAMYYCARLGMITTGYAMDYWGQGTSVTVSSGGGGSGGGGSGGGGSGGGGSDVLMTQTPLSLPVSLGDQASISCRSSQTIVHSTGHTYLEWFLQKPGQSPKLLIYKVSNRFSGVPDRFSGSGSGTDFTLKISRVEAEDLGVYYCFQGSHVPYTFGGGTKLEIKGGGGSFWVLVVVGGVLACYSLLVTVAFIIFWVRSKRSRLLHSDYMNMTPRRPGPTRKHYQPYAPPRDFAAYRSRVKFSRSADAPAYQQGQNQLYNELNLGRREEYDVLDKRRGRDPEMGGKPRRKNPQEGLYNELQKDKMAEAYSEIGMKGERRRGKGHDGLYQGLSTATKDTYDALHMQALPPR

SEQ ID NO: 60 - protein, 272 aa, Artificial sequence
  Anti-AAA-scFv
MNFGLSLVFLALILKGVQCEVQLVESGGDLVKPGGSLKLSCAASGFTFSSYGMSWVRQTPDKRLEWVATISSGGSYIYYPDSVKGRFTISRDNAKNTLYLQMSSLKSEDTAMYYCARLGMITTGYAMDYWGQGTSVTVSSGGGGSGGGGSGGGGSGGGGSDVLMTQTPLSLPVSLGDQASISCRSSQTIVHSTGHTYLEWFLQKPGQSPKLLIYKVSNRFSGVPDRFSGSGSGTDFTLKISRVEAEDLGVYYCFQGSHVPYTFGGGTKLEIK

SEQ ID NO: 61 - protein, 140 aa, Artificial sequence
  Anti-AAA VH
MNFGLSLVFLALILKGVQCEVQLVESGGDLVKPGGSLKLSCAASGFTFSSYGMSWVRQTPDKRLEWVATISSGGSYIYYPDSVKGRFTISRDNAKNTLYLQMSSLKSEDTAMYYCARLGMITTGYAMDYWGQGTSVTVSS

SEQ ID NO: 62 - protein, 112 aa, Artificial sequence
  Anti-AAA VL
DVLMTQTPLSLPVSLGDQASISCRSSQTIVHSTGHTYLEWFLQKPGQSPKLLIYKVSNRFSGVPDRFSGSGSGTDFTLKISRVEAEDLGVYYCFQGSHVPYTFGGGTKLEIK

SEQ ID NO: 63 - protein, 428 aa, Artificial sequence
  Anti-AAA-Fab-heavy chain-CD28ATM-CD28CSD-CD3zSSD fusion
MNFGLSLVFLALILKGVQCEVQLVESGGDLVKPGGSLKLSCAASGFTFSSYGMSWVRQTPDKRLEWVATISSGGSYIYYPDSVKGRFTISRDNAKNTLYLQMSSLKSEDTAMYYCARLGMITTGYAMDYWGQGTSVTVSSASTKGPSVFPLAPSSKSTSGGTAALGCLVKDYFPEPVTVSWNSGALTSGVHTFPAVLQSSGLYSLSSVVTVPSSSLGTQTYICNVNHKPSNTKVDKKVEPKSCGGGGSFWVLVVVGGVLACYSLLVTVAFIIFWVRSKRSRLLHSDYMNMTPRRPGPTRKHYQPYAPPRDFAAYRSRVKFSRSADAPAYQQGQNQLYNELNLGRREEYDVLDKRRGRDPEMGGKPRRKNPQEGLYNELQKDKMAEAYSEIGMKGERRRGKGHDGLYQGLSTATKDTYDALHMQALPPR

SEQ ID NO: 64 - protein, 243 aa, Artificial sequence
  Anti-AAA-Fab heavy chain
MNFGLSLVFLALILKGVQCEVQLVESGGDLVKPGGSLKLSCAASGFTFSSYGMSWVRQTPDKRLEWVATISSGGSYIYYPDSVKGRFTISRDNAKNTLYLQMSSLKSEDTAMYYCARLGMITTGYAMDYWGQGTSVTVSSASTKGPSVFPLAPSSKSTSGGTAALGCLVKDYFPEPVTVSWNSGALTSGVHTFPAVLQSSGLYSLSSVVTVPSSSLGTQTYICNVNHKPSNTKVDKKVEPKSC

SEQ ID NO: 65 - protein, 219 aa, Artificial sequence
  Anti-AAA-Fab light chain
DVLMTQTPLSLPVSLGDQASISCRSSQTIVHSTGHTYLEWFLQKPGQSPKLLIYKVSNRFSGVPDRFSGSGSGTDFTLKISRVEAEDLGVYYCFQGSHVPYTFGGGTKLEIKRTVAAPSVFIFPPSDEQLKSGTASVVCLLNNFYPREAKVQWKVDNALQSGNSQESVTEQDSKDSTYSLSSTLTLSKADYEKHKVYACEVTHQGLSSPVTKSFNRGEC

SEQ ID NO: 66 - protein, 164 aa, Homo sapiens
MKWKALFTAAILQAQLPITEAQSFGLLDPKLCYLLDGILFIYGVILTALFLRVKFSRSADAPAYQQGQNQLYNELNLGRREEYDVLDKRRGRDPEMGGKPQRRKNPQEGLYNELQKDKMAEAYSEIGMKGERRRGKGHDGLYQGLSTATKDTYDALHMQALPPR

SEQ ID NO: 67 - DNA, 492 bp, Homo sapiens
atgaagtggaaggcgcttttcaccgcggccatcctgcaggcacagttgccgattacagaggcacagagctttggcctgctggatcccaaactctgctacctgctggatggaatcctcttcatctatggtgtcattctcactgccttgttcctgagagtgaagttcagcaggagcgcagagccccccgcgtaccagcagggccagaaccagctctataacgagctcaatctaggacgaagagaggagtacgatgttttggacaagagacgtggccgggaccctgagatggggggaaagccgagaaggaagaaccctcaggaaggcctgtacaatgaactgcagaaagataagatggcggaggcctacagtgagattgggatgaaaggcgagcgccggaggggcaaggggcacgatggcctttaccagggtctcagtacagccaccaaggacacctacgacgcccttcacatgcaggccctgccccctcgctaa

SEQ ID NO: 68 - protein, 164 aa, Mus musculus
MKWKVSVLACILHVRFPGAEAQSFGLLDPKLCYLLDGILFIYGVIITALYLRAKFSRSAETAANLQDPNQLYNELNLGRREEYDVLEKKRARDPEMGGKQQRRRNPQEGVYNALQKDKMAEAYSEIGTKGERRRGKGHDGLYQGLSTATKDTYDALHMQTLAPR

SEQ ID NO: 69 - DNA, 495 bp, Mus musculus
atgaagtggaaagtgtctgttctcgcctgcatcctccacgtgcggttcccaggagcagaggcacagagctttggtctgctggatcccaaactctgctacttgctagatggaatcctcttcatctacggagtcatcatcacagccctgtacctgagagcaaaattcagcaggagtgcagagactgctgccaacctgcaggaccccaaccagctctacaatgagctcaatctagggcgaagagaggaatatgacgtcttggagaagaagcgggctcgggatccagagatgggaggcaaacagcagaggaggaggaacccccaggaaggcgtatacaatgcactgcagaaagacaagatggcagaagcctacagtgagatcggcacaaaaggcgagaggcggagaggcaaggggcacgatggcctttaccagggtctcagcactgccaccaaggacacctatgatgccctgcatatgcagaccctggcccctcgctaa

SEQ ID NO: 70 - DNA, 660 bp, Homo sapiens
atgctgcgcctgctgctggcgctgaacctgtttccgagcattcaggtgaccggcaacaaaattctggtgaaacagagcccgatgctggtggcgtatgataacgcggtgaacctgagctgcaaatatagctataacctgtttagccgcgaatttcgcgcgagcctgcataaaggcctggatagcgcggtggaagtgtgcgtggtgtatggcaactatagccagcagctgcaggtgtatagcaaaaccggctttaactgcgatggcaaactgggcaacgaaagcgtgaccttttatctgcagaacctgtatgtgaaccagaccgatatttatttttgcaaaattgaagtgatgtatccgccgccgtatctggataacgaaaaaagcaacggcaccattattcatgtgaaaggcaaacatctgtgcccgagcccgctgtttccgggcccgagcaaaccgttttgggtgctggtggtggtgggcggcgtgctggcgtgctatagcctgctggtgaccgtggcgtttattattttttgggtgcgcagcaaacgcagccgcctgctgcatagcgattatatgaacatgaccccgcgccgcccgggcccgacccgcaaacattatcagccgtatgcgccgccgcgcgattttgcggcgtatcgcagc

SEQ ID NO: 71 - protein, 220 aa, Homo sapiens
MLRLLLALNLFPSIQVTGNKILVKQSPMLVAYDNAVNLSCKYSYNLFSREFRASLHKGLDSAVEVCVVYGNYSQQLQVYSKTGFNCDGKLGNESVTFYLQNLYVNQTDIYFCKIEVMYPPPYLDNEKSNGTIIHVKGKHLCPSPLFPGPSKPFWVLVVVGGVLACYSLLVTVAFIIFWVRSKRSRLLHSDYMNMTPRRPGPTRKHYQPYAPPRDFAAYRS

SEQ ID NO: 72 - DNA, 654 bp, Mus musculus
atgaccctgcgcctgctgtttctggcgctgaacttttttagcgtgcaggtgaccgaaaacaaaattctggtgaaacagagcccgctgctggtggtggatagcaacgaagtgagcctgagctgccgctatagctataacctgctggcgaaagaatttcgcgcgagcctgtataaaggcgtgaacagcgatgtggaagtgtgcgtgggcaacggcaactttacctatcagccgcagtttcgcagcaacgcggaatttaactgcgatggcgattttgataacgaaaccgtgacctttcgcctgtggaacctgcatgtgaaccataccgatatttatttttgcaaaattgaatttatgtatccgccgccgtatctggataacgaacgcagcaacggcaccattattcatattaaagaaaaacatctgtgccatacccagagcagcccgaaactgttttgggcgctggtggtggtggcgggcgtgctgttttgctatggcctgctggtgaccgtggcgctgtgcgtgatttggaccaacagccgccgcaaccgcctgctgcagagcgattatatgaacatgaccccgcgccgcccgggcctgacccgcaaaccgtatcagccgtatgcgccggcgcgcgattttgcggcgtatcgcccg

SEQ ID NO: 73 - protein, 218 aa, Mus musculus
MTLRLLFLALNFFSVQVTENKILVKQSPLLVVDSNEVSLSCRYSYNLLAKEFRASLYKGVNSDVEVCVGNGNFTYQPQFRSNAEFNCDGDFDNETVTFRLWNLHVNHTDIYFCKIEFMYPPPYLDNERSNGTIIHIKEKHLCHTQSSPKLFWALVVVAGVLFCYGLLVTVALCVIWTNSRRNRLLQSDYMNMTPRRPGLTRKPYQPYAPARDFAAYRP

SEQ ID NO: 74 - protein, 4 aa, Artificial sequence
  CD28 YMNM
YMNM

SEQ ID NO: 75 - protein, 4 aa, Artificial sequence
  CD28 PYAP
PYAP

SEQ ID NO: 76 - protein, 21 aa, Artificial sequence
  Signal peptide
ATMGWSCIILFLVATATGVHS

SEQ ID NO: 77 - DNA, 57 bp, Artificial sequence
  Signal peptide DNA sequence
atgggatggagctgtatcatcctcttcttggtagcaacagctaccggtgtgcactcc

SEQ ID NO: 78 - protein, 449 aa, Artificial sequence
  Anti-CD20 (GA101) heavy chain
QVQLVQSGAEVKKPGSSVKVSCKASGYAFSYSWINWVRQAPGQGLEWMGRIFPGDGDTDYNGKFKGRVTITADKSTSTAYMELSSLRSEDTAVYYCARNVFDGYWLVYWGQGTLVTVSSASTKGPSVFPLAPSSKSTSGGTAALGCLVKDYFPEPVTVSWNSGALTSGVHTFPAVLQSSGLYSLSSVVTVPSSSLGTQTYICNVNHKPSNTKVDKKVEPKSCDKTHTCPPCPAPELLGGPSVFLFPPKPKDTLMISRTPEVTCVVVDVSHEDPEVKFNWYVDGVEVHNAKTKPREEQYNSTYRVVSVLTVLHQDWLNGKEYKCKVSNKALPAPIEKTISKAKGQPREPQVYTLPPSRDELTKNQVSLTCLVKGFYPSDIAVEWESNGQPENNYKTTPPVLDSDGSFFLYSKLTVDKSRWQQGNVFSCSVMHEALHNHYTQKSLSLSPGK

SEQ ID NO: 79 - protein, 219 aa, Artificial sequence
  Anti-CD20 (GA101) light chain
DIVMTQTPLSLPVTPGEPASISCRSSKSLLHSNGITYLYWYLQKPGQSPQLLIYQMSNLVSGVPDRFSGSGSGTDFTLKISRVEAEDVGVYYCAQNLELPYTFGGGTKVEIKRTVAAPSVFIFPPSDEQLKSGTASVVCLLNNFYPREAKVQWKVDNALQSGNSQESVTEQDSKDSTYSLSSTLTLSKADYEKHKVYACEVTHQGLSSPVTKSFNRGEC

SEQ ID NO: 80 - protein, 447 aa, Artificial sequence
  Anti-FAP(4B9) PGLALA heavy chain
EVQLLESGGGLVQPGGSLRLSCAASGFTFSSYAMSWVRQAPGKGLEWVSAIIGSGASTYYADSVKGRFTISRDNSKNTLYLQMNSLRAEDTAVYYCAKGWFGGFNYWGQGTLVTVSSASTKGPSVFPLAPSSKSTSGGTAALGCLVKDYFPEPVTVSWNSGALTSGVHTFPAVLQSSGLYSLSSVVTVPSSSLGTQTYICNVNHKPSNTKVDKKVEPKSCDKTHTCPPCPAPEAAGGPSVFLFPPKPKDTLMISRTPEVTCVVVDVSHEDPEVKFNWYVDGVEVHNAKTKPREEQYNSTYRVVSVLTVLHQDWLNGKEYKCKVSNKALGAPIEKTISKAKGQPREPQVYTLPPSRDELTKNQVSLTCLVKGFYPSDIAVEWESNGQPENNYKTTPPVLDSDGSFFLYSKLTVDKSRWQQGNVFSCSVMHEALHNHYTQKSLSLSPGK

SEQ ID NO: 81 - protein, 215 aa, Artificial sequence
  Anti-FAP(4B9) light chain
EIVLTQSPGTLSLSPGERATLSCRASQSVTSSYLAWYQQKPGQAPRLLINVGSRRATGIPDRFSGSGSGTDFTLTISRLEPEDFAVYYCQQGIMLPPTFGQGTKVEIKRTVAAPSVFIFPPSDEQLKSGTASVVCLLNNFYPREAKVQWKVDNALQSGNSQESVTEQDSKDSTYSLSSTLTLSKADYEKHKVYACEVTHQGLSSPVTKSFNRGEC

SEQ ID NO: 82 - protein, 451 aa, Artificial sequence
  Anti-CEA (A5B7) PGLALA heavy chain
EVQLVESGGGLVQPGRSLRLSCAASGFTVSSYWMHWVRQAPGKGLEWVGFIRNKANGGTTEYAASVKGRFTISRDDSKNTLYLQMNSLRAEDTAVYYCARDRGLRFYFDYWGQGTTVTVSSASTKGPSVFPLAPSSKSTSGGTAALGCLVKDYFPEPVTVSWNSGALTSGVHTFPAVLQSSGLYSLSSVVTVPSSSLGTQTYICNVNHKPSNTKVDKKVEPKSCDKTHTCPPCPAPEAAGGPSVFLFPPKPKDTLMISRTPEVTCVVVDVSHEDPEVKFNWYVDGVEVHNAKTKPREEQYNSTYRVVSVLTVLHQDWLNGKEYKCKVSNKALGAPIEKTISKAKGQPREPQVYTLPPSRDELTKNQVSLTCLVKGFYPSDIAVEWESNGQPENNYKTTPPVLDSDGSFFLYSKLTVDKSRWQQGNVFSCSVMHEALHNHYTQKSLSLSPGK

SEQ ID NO: 83 - protein, 223 aa, Artificial sequence
  Anti-CEA (A5B7) light chain
QAVLTQPASLSASPGASASLTCTLRRGINVGAYSIYWYQQKPGSPPQYLLRYKSDSDKQQGSGVSSRFSASKDASANAGILLISGLQSEDEADYYCMIWHSGASAVFGGGTKLTVLRTVAAPSVFIFPPSDEQLKSGTASVVCLLNNFYPREAKVQWKVDNALQSGNSQESVTEQDSKDSTYSLSSTLTLSKADYEKHKVYACEVTHQGLSSPVTKSFNRGEC

SEQ ID NO: 84 - protein, 451 aa, Artificial sequence
  Anti-CEA (T84.66LCHA) PGLALA heavy chain
QVQLVQSGAEVKKPGSSVKVSCKASGFNIKDTYMHWVRQAPGQGLEWMGRIDPANGNSKYVPKFQGRVTITADTSTSTAYMELSSLRSEDTAVYYCAPFGYYVSDYAMAYWGQGTLVTVSSASTKGPSVFPLAPSSKSTSGGTAALGCLVKDYFPEPVTVSWNSGALTSGVHTFPAVLQSSGLYSLSSVVTVPSSSLGTQTYICNVNHKPSNTKVDKKVEPKSCDKTHTCPPCPAPEAAGGPSVFLFPPKPKDTLMISRTPEVTCVVVDVSHEDPEVKFNWYVDGVEVHNAKTKPREEQYNSTYRVVSVLTVLHQDWLNGKEYKCKVSNKALGAPIEKTISKAKGQPREPQVYTLPPSRDELTKNQVSLTCLVKGFYPSDIAVEWESNGQPENNYKTTPPVLDSDGSFFLYSKLTVDKSRWQQGNVFSCSVMHEALHNHYTQKSLSLSPGK

SEQ ID NO: 85 - protein, 218 aa, Artificial sequence
  Anti-CEA (T84.66LCHA) light chain
EIVLTQSPATLSLSPGERATLSCRAGESVDIFGVGFLHWYQQKPGQAPRLLIYRASNRATGIPARFSGSGSGTDFTLTISSLEPEDFAVYYCQQTNEDPYTFGQGTKLEIKRTVAAPSVFIFPPSDEQLKSGTASVVCLLNNFYPREAKVQWKVDNALQSGNSQESVTEQDSKDSTYSLSSTLTLSKADYEKHKVYACEVTHQGLSSPVTKSFNRGEC

SEQ ID NO: 86 - protein, 451 aa, Artificial sequence
  Anti-CEA (CH1A1A98/992F1) PGLALA heavy chain
QVQLVQSGAEVKKPGASVKVSCKASGYTFTEFGMNWVRQAPGQGLEWMGWINTKTGEATYVEEFKGRVTFTTDTSTSTAYMELRSLRSDDTAVYYCARWDFAYYVEAMDYWGQGTTVTVSSASTKGPSVFPLAPSSKSTSGGTAALGCLVKDYFPEPVTVSWNSGALTSGVHTFPAVLQSSGLYSLSSVVTVPSSSLGTQTYICNVNHKPSNTKVDKKVEPKSCDKTHTCPPCPAPEAAGGPSVFLFPPKPKDTLMISRTPEVTCVVVDVSHEDPEVKFNWYVDGVEVHNAKTKPREEQYNSTYRVVSVLTVLHQDWLNGKEYKCKVSNKALGAPIEKTISKAKGQPREPQVCTLPPSRDELTKNQVSLSCAVKGFYPSDIAVEWESNGQPENNYKTTPPVLDSDGSFFLVSKLTVDKSRWQQGNVFSCSVMHEALHNHYTQKSLSLSPGK

SEQ ID NO: 87 - protein, 215 aa, Artificial sequence
  Anti-CEA (CH1A1A98/992F1) light chain
DIQMTQSPSSLSASVGDRVTITCKASAAVGTYVAWYQQKPGKAPKLLIYSASYRKRGVPSRFSGSGSGTDFTLTISSLQPEDFATYYCHQYYTYPLFTFGQGTKLEIKRTVAAPSVFIFPPSDEQLKSGTASVVCLLNNFYPREAKVQWKVDNALQSGNSQESVTEQDSKDSTYSLSSTLTLSKADYEKHKVYACEVTHQGLSSPVTKSFNRGEC

SEQ ID NO: 88 - protein, 449 aa, Artificial sequence
  Anti-CEA (hMN14) PGLALA heavy chain
EVQLVESGGGVVQPGRSLRLSCSASGFDFTTYWMSWVRQAPGKGLEWIGEIHPDSSTINYAPSLKDRFTISRDNAKNTLFLQMDSLRPEDTGVYFCASLYFGFPWFAYWGQGTPVTVSSASTKGPSVFPLAPSSKSTSGGTAALGCLVKDYFPEPVTVSWNSGALTSGVHTFPAVLQSSGLYSLSSVVTVPSSSLGTQTYICNVNHKPSNTKVDKKVEPKSCDKTHTCPPCPAPEAAGGPSVFLFPPKPKDTLMISRTPEVTCVVVDVSHEDPEVKFNWYVDGVEVHNAKTKPREEQYNSTYRVVSVLTVLHQDWLNGKEYKCKVSNKALGAPIEKTISKAKGQPREPQVYTLPPSRDELTKNQVSLTCLVKGFYPSDIAVEWESNGQPENNYKTTPPVLDSDGSFFLYSKLTVDKSRWQQGNVFSCSVMHEALHNHYTQKSLSLSPGK

SEQ ID NO: 89 - protein, 213 aa, Artificial sequence
  Anti-CEA (hMN14) light chain
DIQLTQSPSSLSASVGDRVTITCKASQDVGTSVAWYQQKPGKAPKLLIYWTSTRHTGVPSRFSGSGSGTDFTFTISSLQPEDIATYYCQQYSLYRSFGQGTKVEIKRTVAAPSVFIFPPSDEQLKSGTASVVCLLNNFYPREAKVQWKVDNALQSGNSQESVTEQDSKDSTYSLSSTLTLSKADYEKHKVYACEVTHQGLSSPVTKSFNRGEC

SEQ ID NO: 90 - protein, 451 aa, Artificial sequence
  Anti-TNC (2B10) PGLALA heavy chain
QVQLVQSGAEVKKPGSSVKVSCKASGGTFSSYAISWVRQAPGQGLEWMGGIIPIFGTANYAQKFQGRVTITADKSTSTAYMELSSLRSEDTAVYYCARLYGYAYYGAFDYWGQGTTVTVSSASTKGPSVFPLAPSSKSTSGGTAALGCLVKDYFPEPVTVSWNSGALTSGVHTFPAVLQSSGLYSLSSVVTVPSSSLGTQTYICNVNHKPSNTKVDKKVEPKSCDKTHTCPPCPAPEAAGGPSVFLFPPKPKDTLMISRTPEVTCVVVDVSHEDPEVKFNWYVDGVEVHNAKTKPREEQYNSTYRVVSVLTVLHQDWLNGKEYKCKVSNKALGAPIEKTISKAKGQPREPQVCTLPPSRDELTKNQVSLSCAVKGFYPSDIAVEWESNGQPENNYKTTPPVLDSDGSFFLVSKLTVDKSRWQQGNVFSCSVMHEALHNHYTQKSLSLSPGK

SEQ ID NO: 91 - protein, 214 aa, Artificial sequence
  Anti-TNC (2B10) light chain
DIQMTQSPSSLSASVGDRVTITCRASQGIRNDLGWYQQKPGKAPKRLIYAASSLQSGVPSRFSGSGSGTEFTLTISSLQPEDFATYYCLQNGLQPATFGQGTKVEIKRTVAAPSVFIFPPSDEQLKSGTASVVCLLNNFYPREAKVQWKVDNALQSGNSQESVTEQDSKDSTYSLSSTLTLSKADYEKHKVYACEVTHQGLSSPVTKSFNRGEC

SEQ ID NO: 92 - protein, 449 aa, Artificial sequence
  Anti-HER2 (PER) PG LALA heavy chain 1
EVQLVESGGGLVQPGGSLRLSCAASGFTFTDYTMDWVRQAPGKGLEWVADVNPNSGGSIYNQRFKGRFTLSVDRSKNTLYLQMNSLRAEDTAVYYCARNLGPSFYFDYWGQGTLVTVSSASTKGPSVFPLAPSSKSTSGGTAALGCLVKDYFPEPVTVSWNSGALTSGVHTFPAVLQSSGLYSLSSVVTVPSSSLGTQTYICNVNHKPSNTKVDKKVEPKSCDKTHTCPPCPAPEAAGGPSVFLFPPKPKDTLMISRTPEVTCVVVDVSHEDPEVKFNWYVDGVEVHNAKTKPREEQYNSTYRVVSVLTVLHQDWLNGKEYKCKVSNKALGAPIEKTISKAKGQPREPQVYTLPPSRDELTKNQVSLTCLVKGFYPSDIAVEWESNGQPENNYKTTPPVLDSDGSFFLYSKLTVDKSRWQQGNVFSCSVMHEALHNHYTQKSLSLSPGK

SEQ ID NO: 93 - protein, 214 aa, Artificial sequence
  Anti-HER2 (PER) light chain 1
DIQMTQSPSSLSASVGDRVTITCKASQDVSIGVAWYQQKPGKAPKLLIYSASYRYTGVPSRFSGSGSGTDFTLTISSLQPEDFATYYCQQYYIYPYTFGQGTKVEIKRTVAAPSVFIFPPSDEQLKSGTASVVCLLNNFYPREAKVQWKVDNALQSGNSQESVTEQDSKDSTYSLSSTLTLSKADYEKHKVYACEVTHQGLSSPVTKSFNRGEC

SEQ ID NO: 94 - protein, 449 aa, Artificial sequence; identical to SEQ ID NO: 92
  Anti-HER2 (PER) PG LALA heavy chain 2

SEQ ID NO: 95 - protein, 214 aa, Artificial sequence; identical to SEQ ID NO: 93
  Anti-HER2 (PER) light chain 2

SEQ ID NO: 96 - protein, 372 aa, Artificial sequence
  Anti-WT1 (33F05) PGLALA heavy chain
QVQLQESGPGLVKPSETLSLTCTVSGGSINSYYWSWIRQPPGKGLEWIGYIYYSGSTNYNPSLKSRVTISVDTSKNQFSLKLSSVTAADTAVYYCARSYYEAFDYWGQGTLVTVSSSLGTQTYICNVNHKPSNTKVDKKVEPKSCDKTHTCPPCPAPEAAGGPSVFLFPPKPKDTLMISRTPEVTCVVVDVSHEDPEVKFNWYVDGVEVHNAKTKPREEQYNSTYRVVSVLTVLHQDWLNGKEYKCKVSNKALGAPIEKTISKAKGQPREPQVCTLPPSRDELTKNQVSLSCAVKGFYPSDIAVEWESNGQPENNYKTTPPVLDSDGSFFLVSKLTVDKSRWQQGNVFSCSVMHEALHNHYTQKSLSLSPGK

SEQ ID NO: 97 - protein, 214 aa, Artificial sequence
  Anti-WT1 (33F05) light chain
SSELTQDPAVSVALGQTVRITCQGDSLRSYYASWYQQKPGQAPVLVIYGKNNRPSGIPDRFSGSSSGNTASLTITGAQAEDEADYYCNSPDMNGNAVFGGGTKLTVLRTVAAPSVFIFPPSDEQLKSGTASVVCLLNNFYPREAKVQWKVDNALQSGNSQESVTEQDSKDSTYSLSSTLTLSKADYEKHKVYACEVTHQGLSSPVTKSFNRGEC

SEQ ID NO: 98 - protein, 376 aa, Artificial sequence
  Anti-WT1 (11D06) PGLALA heavy chain
QVQLVQSGAEVKKPGSSVKVSCKASGGTFSSYAISWVRQAPGQGLEWMGGIIPIFGTANYAQKFQGRVTITADKSTSTAYMELSSLRSEDTAVYYCARSIELWWGGFDYWGQGTTVTVSSSLGTQTYICNVNHKPSNTKVDKKVEPKSCDKTHTCPPCPAPEAAGGPSVFLFPPKPKDTLMISRTPEVTCVVVDVSHEDPEVKFNWYVDGVEVHNAKTKPREEQYNSTYRVVSVLTVLHQDWLNGKEYKCKVSNKALGAPIEKTISKAKGQPREPQVCTLPPSRDELTKNQVSLSCAVKGFYPSDIAVEWESNGQPENNYKTTPPVLDSDGSFFLVSKLTVDKSRWQQGNVFSCSVMHEALHNHYTQKSLSLSPGK

SEQ ID NO: 99 - protein, 213 aa, Artificial sequence
  Anti-WT1 (11D06) light chain
DIQMTQSPSTLSASVGDRVTITCRASQSISSWLAWYQQKPGKAPKLLIYDASSLESGVPSRFSGSGSGTEFTLTIGSLQPDDFATYYCQQYEDYTTFGQGTKVEIKRTVAAPSVFIFPPSDEQLKSGTASVVCLLNNFYPREAKVQWKVDNALQSGNSQESVTEQDSKDSTYSLSSTLTLSKADYEKHKVYACEVTHQGLSSPVTKSFNRGEC

SEQ ID NO: 100 - protein, 375 aa, Artificial sequence
  Anti-WT1 (33H09) PGLALA heavy chain
QVQLVQSGAEVKKPGSSVKVSCKASGGTFSSYAISWVRQAPGQGLEWMGGIIPIFGTANYAQKFQGRVTITADKSTSTAYMELSSLRSEDTAVYYCARGSYDLFSLDYWGQGTTVTVSSSLGTQTYICNVNHKPSNTKVDKKVEPKSCDKTHTCPPCPAPEAAGGPSVFLFPPKPKDTLMISRTPEVTCVVVDVSHEDPEVKFNWYVDGVEVHNAKTKPREEQYNSTYRVVSVLTVLHQDWLNGKEYKCKVSNKALGAPIEKTISKAKGQPREPQVCTLPPSRDELTKNQVSLSCAVKGFYPSDIAVEWESNGQPENNYKTTPPVLDSDGSFFLVSKLTVDKSRWQQGNVFSCSVMHEALHNHYTQKSLSLSPGK

SEQ ID NO: 101 - protein, 213 aa, Artificial sequence
  Anti-WT1 (33H09) light chain
DIQMTQSPSTLSASVGDRVTITCRASQSISSWLAWYQQKPGKAPKLLIYDASSLESGVPSRFSGSGSGTEFTLTISSLQPDDFATYYCQQYYDGITFGQGTKVEIKRTVAAPSVFIFPPSDEQLKSGTASVVCLLNNFYPREAKVQWKVDNALQSGNSQESVTEQDSKDSTYSLSSTLTLSKADYEKHKVYACEVTHQGLSSPVTKSFNRGEC

SEQ ID NO: 102 - protein, 375 aa, Artificial sequence
  Anti-WT1 (5E11) PGLALA heavy chain
QVQLVQSGAEVKKPGSSVKVSCKASGGTFSSYAISWVRQAPGQGLEWMGGIIPIFGTANYAQKFQGRVTITADKSTSTAYMELSSLRSEDTAVYYCARSSYDLYSFDYWGQGTTVTVSSSLGTQTYICNVNHKPSNTKVDKKVEPKSCDKTHTCPPCPAPEAAGGPSVFLFPPKPKDTLMISRTPEVTCVVVDVSHEDPEVKFNWYVDGVEVHNAKTKPREEQYNSTYRVVSVLTVLHQDWLNGKEYKCKVSNKALGAPIEKTISKAKGQPREPQVCTLPPSRDELTKNQVSLSCAVKGFYPSDIAVEWESNGQPENNYKTTPPVLDSDGSFFLVSKLTVDKSRWQQGNVFSCSVMHEALHNHYTQKSLSLSPGK

SEQ ID NO: 103 - protein, 215 aa, Artificial sequence
  Anti-WT1 (5E11) light chain
DIQMTQSPSTLSASVGDRVTITCRASQSISSWLAWYQQKPGKAPKLLIYDASSLESGVPSRFSGSGSGTEFTLTISSLQPDDFATYYCQQYSFPPMITFGQGTKVEIKRTVAAPSVFIFPPSDEQLKSGTASVVCLLNNFYPREAKVQWKVDNALQSGNSQESVTEQDSKDSTYSLSSTLTLSKADYEKHKVYACEVTHQGLSSPVTKSFNRGEC

SEQ ID NO: 104 - protein, 5 aa, Artificial sequence
  Anti-CD3 HCDR1 Kabat
TYAMN

SEQ ID NO: 105 - protein, 19 aa, Artificial sequence
  Anti-CD3 HCDR2 Kabat
RIRSKYNNYATYYADSVKG

SEQ ID NO: 106 - protein, 14 aa, Artificial sequence
  Anti-CD3 HCDR3 Kabat
HGNFGNSYVSWFAY

SEQ ID NO: 107 - protein, 14 aa, Artificial sequence
  Anti-CD3 LCDR1 Kabat
GSSTGAVTTSNYAN

SEQ ID NO: 108 - protein, 7 aa, Artificial sequence
  Anti-CD3 LCDR2 Kabat
GTNKRAP

SEQ ID NO: 109 - protein, 9 aa, Artificial sequence
  Anti-CD3 LCDR3 Kabat
ALWYSNLWV